European Patent Application EP 4 183 425 A1, published May 24, 2023. Title: Tissue-occluding agent. Applicant: 3-D Matrix, Ltd. The sequence listing filed with the application follows.

SEQUENCE LISTING (4 sequences)

SEQ ID NO: 1 - protein, 16 aa, synthetic construct
  MOD_RES 1: note = ACETYLATION
RADARADARADARADA

SEQ ID NO: 2 - protein, 13 aa, synthetic construct
  MOD_RES 1: note = ACETYLATION
IEIKIEIKIEIKI

SEQ ID NO: 3 - protein, 12 aa, synthetic construct
  MOD_RES 1: note = ACETYLATION
KLDLKLDLKLDL

SEQ ID NO: 4 - protein, 9 aa, synthetic construct
  MOD_RES 1: note = ACETYLATION
IEIKIEIKI